European Patent Specification EP 3 956 026 B9, published October 4, 2023. Title: p16INK4a INHIBITOR FOR PREVENTING OR TREATING HUNTINGTON'S DISEASE. Applicant: SORBONNE UNIVERSITE CENTRE NATIONAL DE LA RECHERCHE SCIENTIFIQUE (CNRS) ASSISTANCE PUBLIQUE HOPITAUX DE PARIS BUCK INSTITUTE FOR RESEARCH ON AGING. The sequence listing filed with the application follows.

SEQUENCE LISTING (36 sequences)

SEQ ID NO: 1 - DNA, 21 bp, Artificial Sequence
  Primer
agggagtttggtcaatcagaa

SEQ ID NO: 2 - DNA, 21 bp, Artificial Sequence
  Primer
tggagatgaggaatcaaagtt

SEQ ID NO: 3 - DNA, 20 bp, Artificial Sequence
  Primer
ccacttctacgcgtgtgttt

SEQ ID NO: 4 - DNA, 21 bp, Artificial Sequence
  Primer
ccaacgcaccgaatagttacg

SEQ ID NO: 5 - DNA, 18 bp, Artificial Sequence
  Primer
gcgctgcccatcatcatg

SEQ ID NO: 6 - DNA, 20 bp, Artificial Sequence
  Primer
ccctcgtgctgatgctactg

SEQ ID NO: 7 - DNA, 24 bp, Artificial Sequence
  Primer
catcatgacctggtcttctaggaa

SEQ ID NO: 8 - DNA, 21 bp, Artificial Sequence
  Primer
gtgtatagggtcggccatcaa

SEQ ID NO: 9 - DNA, 21 bp, Artificial Sequence
  Primer
cctgccgttgttacctgagag

SEQ ID NO: 10 - DNA, 20 bp, Artificial Sequence
  Primer
ctcaagctccaccacagcct

SEQ ID NO: 11 - DNA, 20 bp, Artificial Sequence
  Primer
agtgttcacgaccagcacca

SEQ ID NO: 12 - DNA, 20 bp, Artificial Sequence
  Primer
ctgggcattccaaagaaccc

SEQ ID NO: 13 - DNA, 21 bp, Artificial Sequence
  Primer
ccagactgaactcattggtgg

SEQ ID NO: 14 - DNA, 21 bp, Artificial Sequence
  Primer
gggaggaccagtcgtggtaaa

SEQ ID NO: 15 - DNA, 21 bp, Artificial Sequence
  Primer
cacgctgcaggctgttgaaag

SEQ ID NO: 16 - DNA, 20 bp, Artificial Sequence
  Primer
caccgaggcactcagaggag

SEQ ID NO: 17 - DNA, 20 bp, Artificial Sequence
  Primer
ccgccattagcgcatcacag

SEQ ID NO: 18 - DNA, 21 bp, Artificial Sequence
  Primer
taattggggctccggctaact

SEQ ID NO: 19 - DNA, 21 bp, Artificial Sequence
  Primer
tgcaggtcgcttccttattcc

SEQ ID NO: 20 - DNA, 20 bp, Artificial Sequence
  Primer
atgctgaggatttggaaagg

SEQ ID NO: 21 - DNA, 20 bp, Artificial Sequence
  Primer
ctcccatctccttcatcaca

SEQ ID NO: 22 - DNA, 18 bp, Artificial Sequence
  Primer
ccaaccgcgagaagatga

SEQ ID NO: 23 - DNA, 20 bp, Artificial Sequence
  Primer
ccagaggcgtacagggatag

SEQ ID NO: 24 - DNA, 18 bp, Artificial Sequence
  Primer
cagcagcatggagccttc

SEQ ID NO: 25 - DNA, 20 bp, Artificial Sequence
  Primer
cgtaactattcggtgcgttg

SEQ ID NO: 26 - DNA, 19 bp, Artificial Sequence
  Primer
ctgcccaacgcaccgaata

SEQ ID NO: 27 - DNA, 20 bp, Artificial Sequence
  Primer
gctgcccatcatcatgacct

SEQ ID NO: 28 - DNA, 20 bp, Artificial Sequence
  Primer
cttcaaggataagggcgaca

SEQ ID NO: 29 - DNA, 21 bp, Artificial Sequence
  Primer
cgactatgcagtgacaggttg

SEQ ID NO: 30 - DNA, 26 bp, Artificial Sequence
  Primer
gctgatataatgatctcttttgcagt

SEQ ID NO: 31 - DNA, 18 bp, Artificial Sequence
  Primer
cataggcatgggccaaaa

SEQ ID NO: 32 - DNA, 21 bp, Artificial Sequence
  Si-RNA targeting exon 1 of CDKN2A
aacgcaccgaatagttacggt

SEQ ID NO: 33 - DNA, 19 bp, Artificial Sequence
  Si-RNA
cugcccaacgcaccgaaua

SEQ ID NO: 34 - DNA, 22 bp, Artificial Sequence
  primer FOSB: Forward
tgacagtgttatcccaagaccc

SEQ ID NO: 35 - DNA, 17 bp, Artificial Sequence
  Primer FOSB: Reverse
ccagcaggacggcatca

SEQ ID NO: 36 - DNA, 18 bp, Artificial Sequence
  Primer: Ryk Reverse
gcccttgggaactactgc